European Patent Specification EP 3 827 085 B1, published December 3, 2025. Title: Neue bakterielle lpp-Mutante und deren Verwendung zur sekretorischen Herstellung von rekombinanten Proteinen. Applicant: Wacker Chemie AG. The sequence listing filed with the application follows.

SEQUENCE LISTING (17 sequences)

SEQ ID NO: 1 - DNA, 237 bp, Escherichia coli
  gene (1)..(237): codierende Sequenz des lpp-Wildtypgens
atgaaagctactaaactggtactgggcgcggtaatcctgggttctactctgctggcaggttgctccagcaacgctaaaatcgatcagctgtcttctgacgttcagactctgaacgctaaagttgaccagctgagcaacgacgtgaacgcaatgcgttccgacgttcaggctgctaaagatgacgcagctcgtgctaaccagcgtctggacaacatggctactaaataccgcaagtaa

SEQ ID NO: 2 - protein, 78 aa, Escherichia coli
  PROPEP (1)..(78): unprozessiertes Lpp-Wildtypprotein
MKATKLVLGAVILGSTLLAGCSSNAKIDQLSSDVQTLNAKVDQLSNDVNAMRSDVQAAKDDAARANQRLDNMATKYRK

SEQ ID NO: 3 - protein, 137 aa, Escherichia coli
  PROPEP (1)..(137): unprozessiertes 2xLpp?-Protein
MKATKLVLGAVILGSTLLAGCSSNAKIDQLSSDVQTLNAKVDQLSNDVNAMRSDVQAAKDDAARANQRLDNMATKYRGGGSSNAKIDQLSSDVQTLNAKVDQLSNDVNAMRSDVQAAKDDAARANQRLDNMATKYRK

SEQ ID NO: 4 - DNA, 90 bp, Klebsiella pneumoniae M5a1
  sig_peptide (1)..(90): Signalpeptid
atgaaaagaaaccgtttttttaatacctcggctgctattgccatttcgattgcattaaatacttttttttgtagcatgcagacgattgct

SEQ ID NO: 5 - DNA, 90 bp, artifiziell
  sig_peptide (1)..(90): artifizielles Signalpeptid
atgaaaagaaaccgtttttttaatacctcggctgctattgccatttcgattgcattacagatcttttttccgtccgcttccgctttcgct

SEQ ID NO: 6 - DNA, 78 bp, artifiziell
  misc_feature (1)..(78): Oligonukleotid lpp-cat-sac-fw
aactttgtgtaatacttgtaacgctacatggagattaactcaatctagagggtattaatagccctgggccaacttttg

SEQ ID NO: 7 - DNA, 78 bp, artifiziell
  misc_feature (1)..(78): Oligonukleotid lpp-cat-sac-rev
taaacggcagacaaaaaaaatggcgcacaatgtgcgccatttttcacttcacaggtactaacactgcttccggtagtc

SEQ ID NO: 8 - DNA, 23 bp, artifiziell
  misc_feature (1)..(23): Oligonukleotid pykF
ctcgcgcagtacgtaaatacttc

SEQ ID NO: 9 - DNA, 21 bp, artifiziell
  misc_feature (1)..(21): Oligonukleotid ynhG2
cgtctttgcttacactcacgc

SEQ ID NO: 10 - DNA, 22 bp, artifiziell
  misc_feature (1)..(22): Oligonukleotid lpp-Allel-fw
atttgtatatcgaagcgccctg

SEQ ID NO: 11 - DNA, 80 bp, artifiziell
  misc_feature (1)..(80): Oligonukleotid lpp-2x-rev2
cattcagggtctgcacatcgctgctcagttgatcaattttggcgttagagcttccgccaccgcggtatttagtagccatg

SEQ ID NO: 12 - DNA, 60 bp, artifiziell
  misc_feature (1)..(60): Oligonukleotid lpp-2x-rev3
acgcattgcattaacatcgtttgacagctgatccactttcgcattcagggtctgcacatc

SEQ ID NO: 13 - DNA, 62 bp, artifiziell
  misc_feature (1)..(62): Oligonukleotid lpp-2x-fw2
gcgcaaatcagcgcctggataatatggcaaccaagtatcgtaaataatagtacctgtgaagt

SEQ ID NO: 14 - DNA, 21 bp, artifiziell
  misc_feature (1)..(21): Oligonukleotid lpp-Allel-rev
cagaagaacagcagaacgttc

SEQ ID NO: 15 - DNA, 75 bp, artifiziell
  misc_feature (1)..(75): Oligonukleotid lpp-2x-fw3
caaacgatgttaatgcaatgcgtagcgatgtgcaggcagcaaaggatgatgcagcacgcgcaaatcagcgcctgg

SEQ ID NO: 16 - DNA, 1005 bp, artifiziell
  misc_feature (293)..(706): Expressionskassette 2xlpp?
atttgtatatcgaagcgccctgatgggcgctttttttatttaatcgataaccagaagcaataaaaaatcaaatcggatttcactatataatctcactttatctaagatgaatccgatggaagcatcctgttttctctcaatttttttatctaaaacccagcgttcgatgcttctttgagcgaacgatcaaaaataagtgccttcccatcaaaaaaatattctcaacataaaaaactttgtgtaatacttgtaacgctacatggagattaactcaatctagagggtattaataatgaaagctactaaactggtactgggcgcggtaatcctgggttctactctgctggcaggttgctccagcaacgctaaaatcgatcagctgtcttctgacgttcagactctgaacgctaaagttgaccagctgagcaacgacgtgaacgcaatgcgttccgacgttcaggctgctaaagatgacgcagctcgtgctaaccagcgtctggacaacatggctactaaataccgcggtggcggaagctctaacgccaaaattgatcaactgagcagcgatgtgcagaccctgaatgcgaaagtggatcagctgtcaaacgatgttaatgcaatgcgtagcgatgtgcaggcagcaaaggatgatgcagcacgcgcaaatcagcgcctggataatatggcaaccaagtatcgtaaataatagtacctgtgaagtgaaaaatggcgcacattgtgcgccattttttttgtctgccgtttaccgctactgcgtcacgcgtaacatattcccttgctctggttcaccattctgcgctgactctactgaaggcgcattgctggctgcgggagttgctccactgctcaccgaaaccggataccctgcccgacgatacaacgctttatcgactaacttctgatctacagccttattgtctttaaattgcgtaaagcctgctggcagtgtgtatggcattgtctgaacgttctgctgttcttctg

SEQ ID NO: 17 - DNA, 1599 bp, artifiziell
  misc_feature (25)..(1549): anti-CD154-Expressionskassette
  sig_peptide (25)..(114): AFA-Signalsequenz
  misc_feature (115)..(777): Leserahmen für HC (VH-CH1)
  sig_peptide (800)..(862): phoA-Signalsequenz
  misc_feature (863)..(1516): Leserahmen für LC (VL-CL)
  misc_feature (1517)..(1546): Linker inkl. His-Tag
acagaattctaaggaggaaattatatgaaaagaaaccgtttttttaatacctcggctgctattgccatttcgattgcattacagatcttttttccgtccgcttccgctttcgctcaggttcagctggtgcagagcggtgccgaagttgttaaaccgggtgcaagcgttaaactgagctgtaaagcaagcggctatatttttaccagctattatatgtattgggtgaaacaggcaccgggtcagggtctggaatggattggtgaaattaatccgagcaatggcgataccaattttaatgaaaaatttaaaagcaaagccaccctgaccgttgataaaagcgcaagcaccgcatatatggaactgagcagcctgcgtagcgaagataccgcagtttattattgtacccgtagtgatggtcgcaatgatatggatagctggggtcagggcaccctggtcaccgttagcagcgcaagcaccaaaggtccgagcgtttttccgctggcaccgagcagcaaaagcaccagcggtggcaccgcagcactgggttgtctggttaaagattattttccggaaccggttacagttagctggaatagcggtgcactgaccagtggtgttcatacctttccggcagttctgcaaagcagcggtctgtatagcctgagcagcgttgttaccgttccgagcagtagcctgggcacccagacctatatttgtaatgttaatcataaaccgagcaacaccaaagtggataaaaaagttgaaccgaaaagctgctaataaccatggagaaaataaagtgaaacaaagcactattgcactggcactcttaccgttactcttcacccctgttaccaaagccgatattgtgctcacccagagtccggcaaccctgagcgttagtccgggtgaacgtgcaaccattagctgtcgtgcaagccagcgtgttagcagcagcacctatagctatatgcattggtatcagcagaaaccgggtcagcctccgaaactgctgattaaatatgcaagcaatctggaaagcggtgttccggcacgttttagcggtagcggtagtggcaccgattttaccctgaccattagcagcgttgaaccggaagattttgccacctattattgtcagcatagctgggaaattcctccgacctttggtggtggcaccaaactcgagattaaacgtaccgttgcagcaccgagcgtgtttatctttccgcctagtgatgaacagctgaaaagcggcaccgcaagcgttgtttgtctgctgaataacttttatccgcgtgaagcaaaagttcagtggaaagttgataatgcactgcaaagcggtaatagccaagaaagcgttaccgaacaggatagcaaagatagcacctatagcctgtcaagcaccctgaccctgagcaaagcagattatgaaaaacacaaagtgtatgcctgcgaagttacccatcagggtctgagcagtccggttacaaaaagttttaatcgtggtgaatgtagctcttctgcccatcaccaccatcaccattaataagcttctagaagcttggctgttttggcggatgagagaagattttcgac